European Patent Application EP 4 800 028 A1, published September 2, 2026. Title: SYSTEME DE CYCLISATION DE PROTEINES RECOMBINANTES POUR LEUR EXPRESSION ET PURIFICATION. Applicant: CENTRE NATIONAL DE LA RECHERCHE SCIENTIFIQUE. The sequence listing filed with the application follows.

SEQUENCE LISTING (15 sequences)

SEQ ID NO: 1 - protein, 5 aa, Synthetic construct
GGGGS

SEQ ID NO: 2 - protein, 10 aa, Synthetic construct
EAAAKEAAAK

SEQ ID NO: 3 - protein, 68 aa, Synthetic construct
DYDMLTEEQKKKLKEDHTLKILLKNNYVREVFKQFTLSNDKIGYLSHYINDPTIVQVIDHIMKTIDDT

SEQ ID NO: 4 - protein, 25 aa, Synthetic construct
DIYTYEKKLIKSIEYITKNKFFDDS

SEQ ID NO: 5 - protein, 83 aa, Synthetic construct
EDVPEYEVKMKRFKGAAYKLRILIENKAPNSKPDRFSPSYNFAENILYINGKLSIPLPRDIVVNAADIKIFHIRKERTLYIYI

SEQ ID NO: 6 - protein, 19 aa, Synthetic construct
SVQIPVVEVDELPEGYDRS

SEQ ID NO: 7 - protein, 253 aa, Synthetic construct
SVQIPVVEVDELPEGYDRSGGGGSLELIVPYNLPLPGGVVPKMLITILGTVKPNANRIALDFQRGNDVAFHFNPRFNENNRRVIVCNTKLDNNWGREERQSVFPFESGKPFKIQVLVEPDHFKVAVNDAHLLQYNHRVKKLNEISKLGISGDIDLTSTSYTMIELGGGGSEDVPEYEVKMKRFKGAAYKLRILIENKAPNSKPDRFSPSYNFAENILYINGKLSIPLPRDIVVNAADIKIFHIRKERTLYIYI

SEQ ID NO: 8 - protein, 473 aa, Synthetic construct
SVQIPVVEVDELPEGYDRSGGGGSLEDNFKHLLGNDNVKRPSEAGALQLQEVDGQMTLVDQHGEKIQLRGMSTHGLQWFPEILNDNAYKALANDWESNMIRLAMYVGENGYASNPELIKSRVIKGIDLAIENDMYVIVDWHVHAPGDPRDPVYAGAEDFFRDIAALYPNNPHIIYELANEPSSNNNGGAGIPNNEEGWNAVKEYADPIVEMLRDSGNADDNIIIVGSPNWSQRPDLAADNPIDDHHTMYTVHFYTGSHAASTESYPPETPNSERGNVMSNTRYALENGVAVFATEWGTSQANGDGGPYFDEADVWIEFLNENNISWANWSLTNKNEVSGAFTPFELGKSNATSLDPGPDQVWVPEELSLSGEYVRARIKGVNYELGGGGSEDVPEYEVKMKRFKGAAYKLRILIENKAPNSKPDRFSPSYNFAENILYINGKLSIPLPRDIVVNAADIKIFHIRKERTLYIYI

SEQ ID NO: 9 - protein, 464 aa, Synthetic construct
DYDMLTEEQKKKLKEDHTLKILLKNNYVREVFKQFTLSNDKIGYLSHYINDPTIVQVIDHIMKTIDDTGGGGSLEDNFKHLLGNDNVKRPSEAGALQLQEVDGQMTLVDQHGEKIQLRGMSTHGLQWFPEILNDNAYKALANDWESNMIRLAMYVGENGYASNPELIKSRVIKGIDLAIENDMYVIVDWHVHAPGDPRDPVYAGAEDFFRDIAALYPNNPHIIYELANEPSSNNNGGAGIPNNEEGWNAVKEYADPIVEMLRDSGNADDNIIIVGSPNWSQRPDLAADNPIDDHHTMYTVHFYTGSHAASTESYPPETPNSERGNVMSNTRYALENGVAVFATEWGTSQANGDGGPYFDEADVWIEFLNENNISWANWSLTNKNEVSGAFTPFELGKSNATSLDPGPDQVWVPEELSLSGEYVRARIKGVNYELGGGGSDIYTYEKKLIKSIEYITKNKFFDDS

SEQ ID NO: 10 - protein, 369 aa, Synthetic construct
SVQIPVVEVDELPEGYDRSLEMTNPYARGPNPTAASLEASAGPFTVRSFTVSRPSGYGAGTVYYPTNAGGTVGAIAIVPGYTARQSSIKWWGPRLASHGFVVITIDTNSTLDQPSSRSSQQMAALRQVASLNGTSSSPIYGKVDTARMGVMGHSMGGGGSLISAANNPSLKAAAPQAPWDSSTNFSSVTVPTLIFACENDSIAPVNSSALPIYDSMSRNAKQFLEINGGSHFCANSGNSNQALIGKKGVAWMKRFMDNDTRYSTFACENPNSTRVSDFRTANCSELEDVPEYEVKMKRFKGAAYKLRILIENKAPNSKPDRFSPSYNFAENILYINGKLSIPLPRDIVVNAADIKIFHIRKERTLYIYI

SEQ ID NO: 11 - protein, 360 aa, Synthetic construct
DYDMLTEEQKKKLKEDHTLKILLKNNYVREVFKQFTLSNDKIGYLSHYINDPTIVQVIDHIMKTIDDTLEMTNPYARGPNPTAASLEASAGPFTVRSFTVSRPSGYGAGTVYYPTNAGGTVGAIAIVPGYTARQSSIKWWGPRLASHGFVVITIDTNSTLDQPSSRSSQQMAALRQVASLNGTSSSPIYGKVDTARMGVMGHSMGGGGSLISAANNPSLKAAAPQAPWDSSTNFSSVTVPTLIFACENDSIAPVNSSALPIYDSMSRNAKQFLEINGGSHFCANSGNSNQALIGKKGVAWMKRFMDNDTRYSTFACENPNSTRVSDFRTANCSELDIYTYEKKLIKSIEYITKNKFFDDS

SEQ ID NO: 12 - protein, 375 aa, Synthetic construct
SVQIPVVEVDELPEGYDRSGGGGSLEMSNPYQRGPNPTRSALTADGPFSVATYTVSRLSVSGFGGGVIYYPTGTSLTFGGIAMSPGYTADASSLAWLGRRLASHGFVVLVINTNSRFDGPDSRASQLSAALNYLRTSSPSAVRARLDANRLAVAGHSMGGGGTLRIAEQNPSLKAAVPLTPWHTDKTFNTSVPVLIVGAEADTVAPVSQHAIPFYQNLPSTTPKVYVELCNASHIAPNSNNAAISVYTISWMKLWVDNDTRYRQFLCNVNDPALCDFRTNNRHCQELGGGGSEDVPEYEVKMKRFKGAAYKLRILIENKAPNSKPDRFSPSYNFAENILYINGKLSIPLPRDIVVNAADIKIFHIRKERTLYIYI

SEQ ID NO: 13 - protein, 366 aa, Synthetic construct
DYDMLTEEQKKKLKEDHTLKILLKNNYVREVFKQFTLSNDKIGYLSHYINDPTIVQVIDHIMKTIDDTGGGGSLEMSNPYQRGPNPTRSALTADGPFSVATYTVSRLSVSGFGGGVIYYPTGTSLTFGGIAMSPGYTADASSLAWLGRRLASHGFVVLVINTNSRFDGPDSRASQLSAALNYLRTSSPSAVRARLDANRLAVAGHSMGGGGTLRIAEQNPSLKAAVPLTPWHTDKTFNTSVPVLIVGAEADTVAPVSQHAIPFYQNLPSTTPKVYVELCNASHIAPNSNNAAISVYTISWMKLWVDNDTRYRQFLCNVNDPALCDFRTNNRHCQELGGGGSDIYTYEKKLIKSIEYITKNKFFDDS

SEQ ID NO: 14 - protein, 126 aa, Synthetic construct
SVQIPVVEVDELPEGYDRSGGGGSLEEAAAKEAAAKELGGGGSEDVPEYEVKMKRFKGAAYKLRILIENKAPNSKPDRFSPSYNFAENILYINGKLSIPLPRDIVVNAADIKIFHIRKERTLYIYI

SEQ ID NO: 15 - protein, 117 aa, Synthetic construct
DYDMLTEEQKKKLKEDHTLKILLKNNYVREVFKQFTLSNDKIGYLSHYINDPTIVQVIDHIMKTIDDTGGGGSLEEAAAKEAAAKELGGGGSDIYTYEKKLIKSIEYITKNKFFDDS